European Patent Application EP 4 653 015 A2, published November 26, 2025. Title: Compositions and Methods of Using Tyrosine Kinase Inhibitors. Applicant: YALE UNIVERSITY. Application EP. The sequence listing filed with the application follows.

SEQUENCE LISTING (21 sequences)

SEQ ID NO: 1 - DNA, 21 bp, synthetic construct
  source 1..21: mol_type = other DNA
accgcagctaggaataatgga

SEQ ID NO: 2 - DNA, 19 bp, synthetic construct
  source 1..19: mol_type = other DNA
accaaaagccttgactccg

SEQ ID NO: 3 - DNA, 25 bp, synthetic construct
  source 1..25: mol_type = other DNA
cctggaggagaagatgccggtagaa

SEQ ID NO: 4 - DNA, 24 bp, synthetic construct
  source 1..24: mol_type = other DNA
ccccagtccagggaggcacctcgg

SEQ ID NO: 5 - DNA, 26 bp, synthetic construct
  source 1..26: mol_type = other DNA
cacttcaaaggtggtcccagagctgc

SEQ ID NO: 6 - DNA, 23 bp, synthetic construct
  source 1..23: mol_type = other DNA
gaccggatcggatccgtcagtcg

SEQ ID NO: 7 - DNA, 22 bp, synthetic construct
  source 1..22: mol_type = other DNA
gtcccggacactggaccaggcc

SEQ ID NO: 8 - DNA, 27 bp, synthetic construct
  source 1..27: mol_type = other DNA
ctccttttcttccagttgcctagccaa

SEQ ID NO: 9 - DNA, 25 bp, synthetic construct
  source 1..25: mol_type = other DNA
gagcaaggccgaggagacgcagcgt

SEQ ID NO: 10 - DNA, 26 bp, synthetic construct
  source 1..26: mol_type = other DNA
gagcctccttctcgtccagctgccgg

SEQ ID NO: 11 - DNA, 20 bp, synthetic construct
  source 1..20: mol_type = other DNA
aggtcttcctggagctgatg

SEQ ID NO: 12 - DNA, 20 bp, synthetic construct
  source 1..20: mol_type = other DNA
acccacagggccttctttac

SEQ ID NO: 13 - DNA, 24 bp, synthetic construct
  source 1..24: mol_type = other DNA
acagcaaattcacttacacagttc

SEQ ID NO: 14 - DNA, 19 bp, synthetic construct
  source 1..19: mol_type = other DNA
ctcattgccttgcgtgttt

SEQ ID NO: 15 - protein, 46 aa, synthetic construct
EGLVKSLPSGSHQGPVIYAQLDHSGGHHSDKINKSESVVYADIRKN

SEQ ID NO: 16 - protein, 47 aa, synthetic construct
EGLVKSPPSAGSHQGPVIYAQLDHSGGHHSGKINKSESVVYADIRKD

SEQ ID NO: 17 - protein, 47 aa, synthetic construct; identical to SEQ ID NO: 16

SEQ ID NO: 18 - protein, 46 aa, synthetic construct
EGLVKSLPSGSHQGPVIYAQLDHSGGHHSDRINKSESVVYADIRKN

SEQ ID NO: 19 - protein, 46 aa, synthetic construct; identical to SEQ ID NO: 15

SEQ ID NO: 20 - protein, 46 aa, synthetic construct
DNSRCSSPSAPVQGPVIYAQLDHSGSKNSSSFHKMEPVVYADIRKN

SEQ ID NO: 21 - protein, 46 aa, synthetic construct
EGLVNSVPARSHQGPVIYAQLDHSGGQHSDKINKSESVVYADIRKN